European Patent Specification EP 3 528 842 B1, published May 27, 2026. Title: RECOMBINANT VECTORS EXPRESSING ANTIGENS OF AVIAN INFLUENZA VIRUS AND USES THEREOF. Applicant: Merial, Inc. The United States of America, as represented by the Secretary of Agriculture Prichard, Joyce Mebatsion, Teshome Swayne, David. The sequence listing filed with the application follows.

SEQUENCE LISTING (28 sequences)

SEQ ID NO: 1 - DNA, 1692 bp, artificial
  DNA encoding H5N2 HA protein in plasmid pHVTIG1SVLPC-HAsyn SbfI and pHVTIG1HHV3gBroSVLPC-HAsyn SbfI
atggaaaagattgtgctgctgtttgctgtgattagcctggtgaagtcagatcagatttgtatcggttaccatgccaataattctactaaacaggtggatacaattatggaaaagaacgtgaccgtgacacacgctcaggacatcctggagagaactcataacgggaagctgtgcgatctgaatggtgtgaaacccctgatcctgaaggactgctctgtggcaggctggctgctgggaaaccccatgtgtgatgagttcatcagagtgcctgaatggtcctacattgtggagagggctaaccctgcaaatgatctgtgctacccaggaaccctgaacgactatgaggaactgaagcacctgctgagccgcatcaaccatttcgaaaagacactgatcatcccccggagctcctggcctaatcacgagactagcctgggagtgtccgcagcttgtccataccagggagcatcttcattctttcgcaacgtggtgtggctgatcaagaaaaatgatgcctaccccaccatcaaaatctcatacaacaacacaaaccgggaagatcttctgatcctgtggggcatccaccattccaacaatgcagccgagcagactaacctgtacaaaaatcctgatacctatgtgtctgtggggacttcaaccctgaaccagcgcctggtgccaaagatcgccactcggtcacaagtgaatgggcagagtggtcgcatggatttcttttggaccatcctgaagccaaacgacgctattcacttcgaaagcaacggcaattttatcgcccccgagtacgcttataagattgtgaagaaaggagacagtaccatcatgaaaagcgagatggaatacgggcactgcaacacaaagtgtcagactcctatcggtgccattaacagtagcatgccattccacaatatccatcccctgacaattggggagtgccccaagtatgtgaaatctaacaagctggtgctggctactggtctgagaaacagccccctgagagagacccggggcctgtttggagcaattgctgggtttattgagggcggatggcagggtatggtggatgggtggtacggttatcaccattccaacgaacaggggtctggttacgctgcagataaagagtccacacagaaggctattgacggagtgactaacaaagtgaacagcatcattgacaagatgaatactcagttcgaggcagtggggagagaatttaacaatctggagagaaggatcgaaaacctgaataagaaaatggaagatggcttcctggacgtgtggacctacaacgcagagctgctggtgctgatggagaatgaaaggacactggattttcacgacagcaacgtgaaaaatctgtatgataaagtgagactgcagctgagggacaacgctaaagaactgggcaatggatgtttcgagttttaccataagtgcgataacgagtgtatggaaagtgtgagaaatggcacatacgactatccaaaatatagcgaggaagcaatcctgaagagggaggaaattagcggcgtgaaactggagtccatcggaacctaccagatcctgtcaatttatagtacagtggcctcctctctggcactggccatcattgtggctgggctgtctctgtggatgtgtagtaacgggagtctgcagtgtaggatttgtatc

SEQ ID NO: 2 - protein, 564 aa, artificial
  H5N2 HA protein in vHVT-501, vHVT-502  and vHVT510
MEKIVLLFAVISLVKSDQICIGYHANNSTKQVDTIMEKNVTVTHAQDILERTHNGKLCDLNGVKPLILKDCSVAGWLLGNPMCDEFIRVPEWSYIVERANPANDLCYPGTLNDYEELKHLLSRINHFEKTLIIPRSSWPNHETSLGVSAACPYQGASSFFRNVVWLIKKNDAYPTIKISYNNTNREDLLILWGIHHSNNAAEQTNLYKNPDTYVSVGTSTLNQRLVPKIATRSQVNGQSGRMDFFWTILKPNDAIHFESNGNFIAPEYAYKIVKKGDSTIMKSEMEYGHCNTKCQTPIGAINSSMPFHNIHPLTIGECPKYVKSNKLVLATGLRNSPLRETRGLFGAIAGFIEGGWQGMVDGWYGYHHSNEQGSGYAADKESTQKAIDGVTNKVNSIIDKMNTQFEAVGREFNNLERRIENLNKKMEDGFLDVWTYNAELLVLMENERTLDFHDSNVKNLYDKVRLQLRDNAKELGNGCFEFYHKCDNECMESVRNGTYDYPKYSEEAILKREEISGVKLESIGTYQILSIYSTVASSLALAIIVAGLSLWMCSNGSLQCRICI

SEQ ID NO: 3 - DNA, 1692 bp, artificial
  DNA encoding mutant H5N2 HA in plasmid pHVTIG1SVMut-HAsyn SbfI (vHVT503)
atggaaaagattgtgctgctgtttgctgtgatttccctggtgaagtccgaccagatttgtattggctaccacgctaataactcaaccaaacaggtggatacaattatggaaaagaacgtgaccgtgacacacgctcaggacatcctggagagaactcataacgggaagctgtgcgatctgaatggtgtgaaacccctgatcctgaaggactgctcagtggcaggctggctgctgggaaaccccatgtgtgatgagttcatcagagtgcctgaatggtcctacattgtggagagggctaaccctgcaaatgatctgtgctacccaggaaccctgaacgactatgaggaactgaagcacctgctgagtcgcatcaaccatttcgaaaagacactgatcatcccccggaacagctggcctaatcacgagacttcactgggcgtgagtgccgcttgtccataccagggagcaagctccttctttcgcaacgtggtgtggctgatcaagaaaaacaatgcctaccccaccatcaaaatctcctacaacaacacaaatcgggaagatcttctgatcctgtggggcatccaccattctaacaatgcagccgagcagactaacctgtacaaaaatcctgacacctatgtgagcgtggggacttccaccctgaaccagcgcctggtgccaaagatcgccactcggtctcaggtgaacgggcagaatggtcgcatggatttcttttggaccatcctgaagccaaatgacgctattcacttcgaatccaacggcaattttatcgcccccgagtacgcttataagattgtgaagaaaggagactctaccatcatgaaatcagagatggaatacgggcactgcaacacaaagtgtcagactcctatcggtgccattaactcttcaatgccattccacaatatccatcccctgacaattggggagtgccccaagtatgtgaaatcaaacaagctggtgctggctactggtctgaggaatagtcctctgcgcgaaacccggggcctgtttggagcaattgctggttttattgagggcggatggcagggtatggtggatgggtggtacggttatcaccatagtaacgaacaggggagcggttacgctgcagataaagagtctacacagaaggctattgacggagtgactaacaaagtgaacagcatcattgacaagatgaacactcagttcgaggcagtggggagagaatttaacaatctggagagaaggatcgaaaacctgaataagaaaatggaagatggcttcctggacgtgtggacctacaacgcagagctgctggtgctgatggagaatgaaaggacactggattttcacgacagcaacgtgaaaaatctgtatgataaagtgagactgcagctgagggacaacgctaaagaactgggcaatggatgtttcgagttttaccataagtgcgataacgagtgtatggaaagcgtgagaaatggcacatacgactatccaaaatattccgaggaagcaatcctgaagagggaggaaatttccggcgtgaaactggagtctatcggaacctaccagatcctgtccatttattctacagtggccagtagcctggcactggccatcattgtggctggtctgtctctgtggatgtgttcaaacggtagtctgcagtgtagaatctgtatc

SEQ ID NO: 4 - protein, 564 aa, artificial
  mutant H5N2 HA in vHVT503
MEKIVLLFAVISLVKSDQICIGYHANNSTKQVDTIMEKNVTVTHAQDILERTHNGKLCDLNGVKPLILKDCSVAGWLLGNPMCDEFIRVPEWSYIVERANPANDLCYPGTLNDYEELKHLLSRINHFEKTLIIPRNSWPNHETSLGVSAACPYQGASSFFRNVVWLIKKNNAYPTIKISYNNTNREDLLILWGIHHSNNAAEQTNLYKNPDTYVSVGTSTLNQRLVPKIATRSQVNGQNGRMDFFWTILKPNDAIHFESNGNFIAPEYAYKIVKKGDSTIMKSEMEYGHCNTKCQTPIGAINSSMPFHNIHPLTIGECPKYVKSNKLVLATGLRNSPLRETRGLFGAIAGFIEGGWQGMVDGWYGYHHSNEQGSGYAADKESTQKAIDGVTNKVNSIIDKMNTQFEAVGREFNNLERRIENLNKKMEDGFLDVWTYNAELLVLMENERTLDFHDSNVKNLYDKVRLQLRDNAKELGNGCFEFYHKCDNECMESVRNGTYDYPKYSEEAILKREEISGVKLESIGTYQILSIYSTVASSLALAIIVAGLSLWMCSNGSLQCRICI

SEQ ID NO: 5 - DNA, 368 bp, artificial
  SV40 promoter
caattcgagctcggtacagcttggctgtggaatgtgtgtcagttagggtgtggaaagtccccaggctccccagcaggcagaagtatgcaaagcatgcatctcaattagtcagcaaccaggtgtggaaagtccccaggctccccagcaggcagaagtatgcaaagcatgcatctcaattagtcagcaaccatagtcccgcccctaactccgcccatcccgcccctaactccgcccagttccgcccattctccgccccatggctgactaattttttttatttatgcagaggccgaggccgcctcggcctctgagctattccagaagtagtgaggaggcttttttggaggcctaggcttttgcaaaaagct

SEQ ID NO: 6 - DNA, 478 bp, artificial
  HHV3gB promoter
ttatatcttctgattgtgtgggctctacttgtaaactctcaaaaaacgagcttggagagaccgacacaaccgccgtaacaaacaaagaaaatatgcataaaaagcataaccacacccccgtaacggatgttatgaaaacgccgggtccgttgaatccggagccagccgctgcattagggtgtatagaagagaaaaaacgtctgaatcgtagattacgacggtattctggtcgatccctgtttctccactttgaataatagccacaaggggacatgtttcttcgtacgttaaataaatgccgtctaagggtccgtgggaactgcctatacctttaggttgagacgtgcacccgcgtggatccttacctagacggtcaacgcgacataaccgcacctccccacaatggaaaacagaggtgaatagtgtggttgcaaacacaagctccctaatatatttccaggcaagtctctgaattccc

SEQ ID NO: 7 - DNA, 154 bp, artificial
  Synthetic Poly A
aataaaatatctttattttcattacatctgtgtgttggttttttgtgtgaatcgatagtactaacatacgctctccatcaaaacaaaacgaaacaaaacaaactagcaaaataggctgtccccagtgcaagtgcaggtgccagaacatttctct

SEQ ID NO: 8 - DNA, 4359 bp, artificial
  Nucleotide sequence of donor plasmid:  pHVTIG1SVLPC-HAsyn SbfI
  Flanking Arms (1)..(832)
  SV40 Promoter (853)..(1220)
  HA H5N2 (1236)..(2930)
  Synthetic Poly A (2945)..(3098)
  Flanking Arms (3119)..(4359)
ctcgaggatacatccaaagaggttgagtattctctctacacttcttgttaaatggaaagtgcatttgcttgttcttacaatcggcccgagtctcgttcacagcgcctcgttcacacttaaaccacaaatagtctacaggctatatgggagccagactgaaactcacatatgactaatattcgggggtgttagtcacgtgtagcccattgtgtgcatataacgatgttggacgcgtccttattcgcggtgtacttgatactatggcagcgagcatgggatattcatcctcgtcatcgttaacatctctacgggttcagaatgtttggcatgtcgtcgatcctttgcccatcgttgcaaattacaagtccgatcgccatgaccgcgataagcctgtaccatgtggcattagggtgacatctcgatcatacattataagaccaacgtgcgagtcttccaaagacctgcacgccttcttcttcggattgtcaacgggttcttcagaatctatgcccatatctggcgttgagaccattgtgcgtttaatgaacaataaagcggcatgccatggaaaggagggctgcagatctccattttctcacgccactatcctggacgctgtagacgataattataccatgaatatagagggggtatgtttccactgccactgtgatgataagttttctccagattgttggatatctgcattttctgctgccgaacaaacttcatcgctatgcaaagagatgcgtgtgtacacgcgccgttgagtatacgggaaactaaatgttcatagaggtctttgggctatatgttattaaataaaataattgtcgaccctgcaggtcgacccaattcgagctcggtacagcttggctgtggaatgtgtgtcagttagggtgtggaaagtccccaggctccccagcaggcagaagtatgcaaagcatgcatctcaattagtcagcaaccaggtgtggaaagtccccaggctccccagcaggcagaagtatgcaaagcatgcatctcaattagtcagcaaccatagtcccgcccctaactccgcccatcccgcccctaactccgcccagttccgcccattctccgccccatggctgactaattttttttatttatgcagaggccgaggccgcctcggcctctgagctattccagaagtagtgaggaggcttttttggaggcctaggcttttgcaaaaagctcccggggcggccgccatggaaaagattgtgctgctgtttgctgtgattagcctggtgaagtcagatcagatttgtatcggttaccatgccaataattctactaaacaggtggatacaattatggaaaagaacgtgaccgtgacacacgctcaggacatcctggagagaactcataacgggaagctgtgcgatctgaatggtgtgaaacccctgatcctgaaggactgctctgtggcaggctggctgctgggaaaccccatgtgtgatgagttcatcagagtgcctgaatggtcctacattgtggagagggctaaccctgcaaatgatctgtgctacccaggaaccctgaacgactatgaggaactgaagcacctgctgagccgcatcaaccatttcgaaaagacactgatcatcccccggagctcctggcctaatcacgagactagcctgggagtgtccgcagcttgtccataccagggagcatcttcattctttcgcaacgtggtgtggctgatcaagaaaaatgatgcctaccccaccatcaaaatctcatacaacaacacaaaccgggaagatcttctgatcctgtggggcatccaccattccaacaatgcagccgagcagactaacctgtacaaaaatcctgatacctatgtgtctgtggggacttcaaccctgaaccagcgcctggtgccaaagatcgccactcggtcacaagtgaatgggcagagtggtcgcatggatttcttttggaccatcctgaagccaaacgacgctattcacttcgaaagcaacggcaattttatcgcccccgagtacgcttataagattgtgaagaaaggagacagtaccatcatgaaaagcgagatggaatacgggcactgcaacacaaagtgtcagactcctatcggtgccattaacagtagcatgccattccacaatatccatcccctgacaattggggagtgccccaagtatgtgaaatctaacaagctggtgctggctactggtctgagaaacagccccctgagagagacccggggcctgtttggagcaattgctgggtttattgagggcggatggcagggtatggtggatgggtggtacggttatcaccattccaacgaacaggggtctggttacgctgcagataaagagtccacacagaaggctattgacggagtgactaacaaagtgaacagcatcattgacaagatgaatactcagttcgaggcagtggggagagaatttaacaatctggagagaaggatcgaaaacctgaataagaaaatggaagatggcttcctggacgtgtggacctacaacgcagagctgctggtgctgatggagaatgaaaggacactggattttcacgacagcaacgtgaaaaatctgtatgataaagtgagactgcagctgagggacaacgctaaagaactgggcaatggatgtttcgagttttaccataagtgcgataacgagtgtatggaaagtgtgagaaatggcacatacgactatccaaaatatagcgaggaagcaatcctgaagagggaggaaattagcggcgtgaaactggagtccatcggaacctaccagatcctgtcaatttatagtacagtggcctcctctctggcactggccatcattgtggctgggctgtctctgtggatgtgtagtaacgggagtctgcagtgtaggatttgtatctgagcggccgcgatatcaataaaatatctttattttcattacatctgtgtgttggttttttgtgtgaatcgatagtactaacatacgctctccatcaaaacaaaacgaaacaaaacaaactagcaaaataggctgtccccagtgcaagtgcaggtgccagaacatttctcttctagacctgcagggaattcgtttaatgttagtttattcaatgcattggttgcaaatattcattacttctccaatcccaggtcattctttagcgagatgatgttatgacattgctgtgaaaattactacaggatatatttttaagatgcaggagtaacaatgtgcatagtaggcgtagttatcgcagacgtgcaacgcttcgcatttgagttaccgaagtgcccaacagtgctgcggttatggtttatgcgcacagaatccatgcatgtcctaattgaaccatccgatttttcttttaatcgcgatcgttgtttgggcaactgcgttatttcagatctaaaaaatttaccctttatgaccatcacatctctctggctcataccccgcttggataagatatcatgtagattccgccctaagaaatgcaaactaacattattgtcggttccatatacacttccatcttgtccttcgaaaataacaaactcgcgcaatagaccgtccgtacatgcatggccgatgtgtgtcaacatcattggtctgctagatcccgatgggacgaatcgtacagtcgtcgctccagcattggcaaaaatccccagataccctccatgcggcaaatctaaattgcgaccccgaagagactgcaccaaagtcttatcgacgcacgctgatttttttgaacagcgggagcccattatcttcagtggagcgtagacgggcgaggctaattatgtgacatagcaacactgcatgtatgtttttataaatcaataagagtacataatttattacgtatcatttccgtttgtaatatactgtatacatcatccacactattagtcagcactagcgcgcgggcgcacgttacaatagcagcgtgcccgttatctatattgtccgatatttacacataacatttcatcgacatgattaaatacctaagtactgcacacagatgtttaatgtatatcgtcatataaattatatcgctaggacagacccaaacgacctttatcccaaacagtcagatcctcttctcaagtgtcgatttctgttatggaatatgcataccctggcccagaaattgcacgcacgagcgtagtgaatgcgtcattggttttacatttaaaggctaaatgcacaaattctttagacgacagcacatcgttaaatagcatctctagcgttcttatgaatgctaagcattggagtcctcctggtcggccacaataacagctgagtatcataccctgagctc

SEQ ID NO: 9 - DNA, 4852 bp, artificial
  Nucleotide sequence of donor plasmid:  pHVTIG1HHV3gBroSVLPC-HAsyn SbfI
  Flanking Arms (1)..(1241)
  HHV3gB promoter (1271)..(1748)
  SV40 Promoter (1755)..(2122)
  HA H5N2 (2138)..(3832)
  Synthetic Poly A (3847)..(4000)
  Flanking Arms (4021)..(4852)
gagctcagggtatgatactcagctgttattgtggccgaccaggaggactccaatgcttagcattcataagaacgctagagatgctatttaacgatgtgctgtcgtctaaagaatttgtgcatttagcctttaaatgtaaaaccaatgacgcattcactacgctcgtgcgtgcaatttctgggccagggtatgcatattccataacagaaatcgacacttgagaagaggatctgactgtttgggataaaggtcgtttgggtctgtcctagcgatataatttatatgacgatatacattaaacatctgtgtgcagtacttaggtatttaatcatgtcgatgaaatgttatgtgtaaatatcggacaatatagataacgggcacgctgctattgtaacgtgcgcccgcgcgctagtgctgactaatagtgtggatgatgtatacagtatattacaaacggaaatgatacgtaataaattatgtactcttattgatttataaaaacatacatgcagtgttgctatgtcacataattagcctcgcccgtctacgctccactgaagataatgggctcccgctgttcaaaaaaatcagcgtgcgtcgataagactttggtgcagtctcttcggggtcgcaatttagatttgccgcatggagggtatctggggatttttgccaatgctggagcgacgactgtacgattcgtcccatcgggatctagcagaccaatgatgttgacacacatcggccatgcatgtacggacggtctattgcgcgagtttgttattttcgaaggacaagatggaagtgtatatggaaccgacaataatgttagtttgcatttcttagggcggaatctacatgatatcttatccaagcggggtatgagccagagagatgtgatggtcataaagggtaaattttttagatctgaaataacgcagttgcccaaacaacgatcgcgattaaaagaaaaatcggatggttcaattaggacatgcatggattctgtgcgcataaaccataaccgcagcactgttgggcacttcggtaactcaaatgcgaagcgttgcacgtctgcgataactacgcctactatgcacattgttactcctgcatcttaaaaatatatcctgtagtaattttcacagcaatgtcataacatcatctcgctaaagaatgacctgggattggagaagtaatgaatatttgcaaccaatgcattgaataaactaacattaaacgaattccctgcaggtcgaggccgcccgggttatatcttctgattgtgtgggctctacttgtaaactctcaaaaaacgagcttggagagaccgacacaaccgccgtaacaaacaaagaaaatatgcataaaaagcataaccacacccccgtaacggatgttatgaaaacgccgggtccgttgaatccggagccagccgctgcattagggtgtatagaagagaaaaaacgtctgaatcgtagattacgacggtattctggtcgatccctgtttctccactttgaataatagccacaaggggacatgtttcttcgtacgttaaataaatgccgtctaagggtccgtgggaactgcctatacctttaggttgagacgtgcacccgcgtggatccttacctagacggtcaacgcgacataaccgcacctccccacaatggaaaacagaggtgaatagtgtggttgcaaacacaagctccctaatatatttccaggcaagtctctgaattccctcgacccaattcgagctcggtacagcttggctgtggaatgtgtgtcagttagggtgtggaaagtccccaggctccccagcaggcagaagtatgcaaagcatgcatctcaattagtcagcaaccaggtgtggaaagtccccaggctccccagcaggcagaagtatgcaaagcatgcatctcaattagtcagcaaccatagtcccgcccctaactccgcccatcccgcccctaactccgcccagttccgcccattctccgccccatggctgactaattttttttatttatgcagaggccgaggccgcctcggcctctgagctattccagaagtagtgaggaggcttttttggaggcctaggcttttgcaaaaagctcccggggcggccgccatggaaaagattgtgctgctgtttgctgtgattagcctggtgaagtcagatcagatttgtatcggttaccatgccaataattctactaaacaggtggatacaattatggaaaagaacgtgaccgtgacacacgctcaggacatcctggagagaactcataacgggaagctgtgcgatctgaatggtgtgaaacccctgatcctgaaggactgctctgtggcaggctggctgctgggaaaccccatgtgtgatgagttcatcagagtgcctgaatggtcctacattgtggagagggctaaccctgcaaatgatctgtgctacccaggaaccctgaacgactatgaggaactgaagcacctgctgagccgcatcaaccatttcgaaaagacactgatcatcccccggagctcctggcctaatcacgagactagcctgggagtgtccgcagcttgtccataccagggagcatcttcattctttcgcaacgtggtgtggctgatcaagaaaaatgatgcctaccccaccatcaaaatctcatacaacaacacaaaccgggaagatcttctgatcctgtggggcatccaccattccaacaatgcagccgagcagactaacctgtacaaaaatcctgatacctatgtgtctgtggggacttcaaccctgaaccagcgcctggtgccaaagatcgccactcggtcacaagtgaatgggcagagtggtcgcatggatttcttttggaccatcctgaagccaaacgacgctattcacttcgaaagcaacggcaattttatcgcccccgagtacgcttataagattgtgaagaaaggagacagtaccatcatgaaaagcgagatggaatacgggcactgcaacacaaagtgtcagactcctatcggtgccattaacagtagcatgccattccacaatatccatcccctgacaattggggagtgccccaagtatgtgaaatctaacaagctggtgctggctactggtctgagaaacagccccctgagagagacccggggcctgtttggagcaattgctgggtttattgagggcggatggcagggtatggtggatgggtggtacggttatcaccattccaacgaacaggggtctggttacgctgcagataaagagtccacacagaaggctattgacggagtgactaacaaagtgaacagcatcattgacaagatgaatactcagttcgaggcagtggggagagaatttaacaatctggagagaaggatcgaaaacctgaataagaaaatggaagatggcttcctggacgtgtggacctacaacgcagagctgctggtgctgatggagaatgaaaggacactggattttcacgacagcaacgtgaaaaatctgtatgataaagtgagactgcagctgagggacaacgctaaagaactgggcaatggatgtttcgagttttaccataagtgcgataacgagtgtatggaaagtgtgagaaatggcacatacgactatccaaaatatagcgaggaagcaatcctgaagagggaggaaattagcggcgtgaaactggagtccatcggaacctaccagatcctgtcaatttatagtacagtggcctcctctctggcactggccatcattgtggctgggctgtctctgtggatgtgtagtaacgggagtctgcagtgtaggatttgtatctgagcggccgcgatatcaataaaatatctttattttcattacatctgtgtgttggttttttgtgtgaatcgatagtactaacatacgctctccatcaaaacaaaacgaaacaaaacaaactagcaaaataggctgtccccagtgcaagtgcaggtgccagaacatttctcttctagacctgcagggtcgacaattattttatttaataacatatagcccaaagacctctatgaacatttagtttcccgtatactcaacggcgcgtgtacacacgcatctctttgcatagcgatgaagtttgttcggcagcagaaaatgcagatatccaacaatctggagaaaacttatcatcacagtggcagtggaaacataccccctctatattcatggtataattatcgtctacagcgtccaggatagtggcgtgagaaaatggagatctgcagccctcctttccatggcatgccgctttattgttcattaaacgcacaatggtctcaacgccagatatgggcatagattctgaagaacccgctgacaatccgaagaagaaggcgtgcaggtctttggaagactcgcacgttggtcttataatgtatgatcgagatgtcaccctaatgccacatggtacaggcttatcgcggtcatggcgatcggacttgtaatttgcaacgatgggcaaaggatcgacgacatgccaaacattctgaacccgtagagatgttaacgatgacgaggatgaatatcccatgctcgctgccatagtatcaagtacaccgcgaataaggacgcgtccaacatcgttatatgcacacaatgggctacacgtgactaacacccccgaatattagtcatatgtgagtttcagtctggctcccatatagcctgtagactatttgtggtttaagtgtgaacgaggcgctgtgaacgagactcgggccgattgtaagaacaagcaaatgcactttccatttaacaagaagtgtagagagaatactcaacctctttggatgtatcctcgag

SEQ ID NO: 10 - DNA, 4359 bp, artificial
  Nucleotide sequence of donor plasmid:  pHVTIG1SVMut-HAsyn SbfI
  Flanking Arms (1)..(832)
  SV40 Promoter (853)..(1220)
  Mut-HA H5N2 (1236)..(2930)
  Synthetic Poly A (2945)..(3098)
  Flanking Arms (3119)..(4359)
ctcgaggatacatccaaagaggttgagtattctctctacacttcttgttaaatggaaagtgcatttgcttgttcttacaatcggcccgagtctcgttcacagcgcctcgttcacacttaaaccacaaatagtctacaggctatatgggagccagactgaaactcacatatgactaatattcgggggtgttagtcacgtgtagcccattgtgtgcatataacgatgttggacgcgtccttattcgcggtgtacttgatactatggcagcgagcatgggatattcatcctcgtcatcgttaacatctctacgggttcagaatgtttggcatgtcgtcgatcctttgcccatcgttgcaaattacaagtccgatcgccatgaccgcgataagcctgtaccatgtggcattagggtgacatctcgatcatacattataagaccaacgtgcgagtcttccaaagacctgcacgccttcttcttcggattgtcaacgggttcttcagaatctatgcccatatctggcgttgagaccattgtgcgtttaatgaacaataaagcggcatgccatggaaaggagggctgcagatctccattttctcacgccactatcctggacgctgtagacgataattataccatgaatatagagggggtatgtttccactgccactgtgatgataagttttctccagattgttggatatctgcattttctgctgccgaacaaacttcatcgctatgcaaagagatgcgtgtgtacacgcgccgttgagtatacgggaaactaaatgttcatagaggtctttgggctatatgttattaaataaaataattgtcgaccctgcaggtcgacccaattcgagctcggtacagcttggctgtggaatgtgtgtcagttagggtgtggaaagtccccaggctccccagcaggcagaagtatgcaaagcatgcatctcaattagtcagcaaccaggtgtggaaagtccccaggctccccagcaggcagaagtatgcaaagcatgcatctcaattagtcagcaaccatagtcccgcccctaactccgcccatcccgcccctaactccgcccagttccgcccattctccgccccatggctgactaattttttttatttatgcagaggccgaggccgcctcggcctctgagctattccagaagtagtgaggaggcttttttggaggcctaggcttttgcaaaaagctcccggggcggccgccatggaaaagattgtgctgctgtttgctgtgatttccctggtgaagtccgaccagatttgtattggctaccacgctaataactcaaccaaacaggtggatacaattatggaaaagaacgtgaccgtgacacacgctcaggacatcctggagagaactcataacgggaagctgtgcgatctgaatggtgtgaaacccctgatcctgaaggactgctcagtggcaggctggctgctgggaaaccccatgtgtgatgagttcatcagagtgcctgaatggtcctacattgtggagagggctaaccctgcaaatgatctgtgctacccaggaaccctgaacgactatgaggaactgaagcacctgctgagtcgcatcaaccatttcgaaaagacactgatcatcccccggaacagctggcctaatcacgagacttcactgggcgtgagtgccgcttgtccataccagggagcaagctccttctttcgcaacgtggtgtggctgatcaagaaaaacaatgcctaccccaccatcaaaatctcctacaacaacacaaatcgggaagatcttctgatcctgtggggcatccaccattctaacaatgcagccgagcagactaacctgtacaaaaatcctgacacctatgtgagcgtggggacttccaccctgaaccagcgcctggtgccaaagatcgccactcggtctcaggtgaacgggcagaatggtcgcatggatttcttttggaccatcctgaagccaaatgacgctattcacttcgaatccaacggcaattttatcgcccccgagtacgcttataagattgtgaagaaaggagactctaccatcatgaaatcagagatggaatacgggcactgcaacacaaagtgtcagactcctatcggtgccattaactcttcaatgccattccacaatatccatcccctgacaattggggagtgccccaagtatgtgaaatcaaacaagctggtgctggctactggtctgaggaatagtcctctgcgcgaaacccggggcctgtttggagcaattgctggttttattgagggcggatggcagggtatggtggatgggtggtacggttatcaccatagtaacgaacaggggagcggttacgctgcagataaagagtctacacagaaggctattgacggagtgactaacaaagtgaacagcatcattgacaagatgaacactcagttcgaggcagtggggagagaatttaacaatctggagagaaggatcgaaaacctgaataagaaaatggaagatggcttcctggacgtgtggacctacaacgcagagctgctggtgctgatggagaatgaaaggacactggattttcacgacagcaacgtgaaaaatctgtatgataaagtgagactgcagctgagggacaacgctaaagaactgggcaatggatgtttcgagttttaccataagtgcgataacgagtgtatggaaagcgtgagaaatggcacatacgactatccaaaatattccgaggaagcaatcctgaagagggaggaaatttccggcgtgaaactggagtctatcggaacctaccagatcctgtccatttattctacagtggccagtagcctggcactggccatcattgtggctggtctgtctctgtggatgtgttcaaacggtagtctgcagtgtagaatctgtatctgagcggccgcgatatcaataaaatatctttattttcattacatctgtgtgttggttttttgtgtgaatcgatagtactaacatacgctctccatcaaaacaaaacgaaacaaaacaaactagcaaaataggctgtccccagtgcaagtgcaggtgccagaacatttctcttctagacctgcagggaattcgtttaatgttagtttattcaatgcattggttgcaaatattcattacttctccaatcccaggtcattctttagcgagatgatgttatgacattgctgtgaaaattactacaggatatatttttaagatgcaggagtaacaatgtgcatagtaggcgtagttatcgcagacgtgcaacgcttcgcatttgagttaccgaagtgcccaacagtgctgcggttatggtttatgcgcacagaatccatgcatgtcctaattgaaccatccgatttttcttttaatcgcgatcgttgtttgggcaactgcgttatttcagatctaaaaaatttaccctttatgaccatcacatctctctggctcataccccgcttggataagatatcatgtagattccgccctaagaaatgcaaactaacattattgtcggttccatatacacttccatcttgtccttcgaaaataacaaactcgcgcaatagaccgtccgtacatgcatggccgatgtgtgtcaacatcattggtctgctagatcccgatgggacgaatcgtacagtcgtcgctccagcattggcaaaaatccccagataccctccatgcggcaaatctaaattgcgaccccgaagagactgcaccaaagtcttatcgacgcacgctgatttttttgaacagcgggagcccattatcttcagtggagcgtagacgggcgaggctaattatgtgacatagcaacactgcatgtatgtttttataaatcaataagagtacataatttattacgtatcatttccgtttgtaatatactgtatacatcatccacactattagtcagcactagcgcgcgggcgcacgttacaatagcagcgtgcccgttatctatattgtccgatatttacacataacatttcatcgacatgattaaatacctaagtactgcacacagatgtttaatgtatatcgtcatataaattatatcgctaggacagacccaaacgacctttatcccaaacagtcagatcctcttctcaagtgtcgatttctgttatggaatatgcataccctggcccagaaattgcacgcacgagcgtagtgaatgcgtcattggttttacatttaaaggctaaatgcacaaattctttagacgacagcacatcgttaaatagcatctctagcgttcttatgaatgctaagcattggagtcctcctggtcggccacaataacagctgagtatcataccctgagctc

SEQ ID NO: 11 - DNA, 124 bp, artificial
  vaccinia H6 promoter
ttctttattctatacttaaaaagtgaaaataaatacaaaggttcttgagggttgtgttaaattgaaagcgagaaataatcataaattatttcattatcgcgatatccgttaagtttgtatcgta

SEQ ID NO: 12 - DNA, 4754 bp, artificial
  Nucleotide sequence of donor plasmid  pF8 H6pLPC-HA H5N2
  Flanking Arms (1)..(1429)
  H6 Promoter (1516)..(1639)
  HA H5N2 (1649)..(3343)
  Flanking Arms (3379)..(4754)
gaccctttacaagaataaaagaagaaacaactgtgaaatagtttataaatgtaattcgtatgcagaaaacgataatatattttggtatgagaaatctaaaggagacatagtttgtatagacatgcgctcttccgatgagatattcgatgcttttctaatgtatcatatagctacaagatatgcctatcatgatgatgatatatatctacaaatagtgttatattattctaataatcaaaatgttatatcttatattacgaaaaataaatacgttaagtatataagaaataaaactagagacgatattcataaagtaaaaatattagctctagaagactttacaacggaagaaatatattgttggattagtaatatataacagcgtagctgcacggttttgatcattttccaacaatataaaccaatgaaggaggacgactcatcaaacataaataacattcacggaaaatattcagtatcagatttatcacaagatgattatgttattgaatgtatagacggatcttttgattcgatcaagtatagagatataaaggttataataatgaagaataacggttacgttaattgtagtaaattatgtaaaatgcggaataaatacttttctagatggttgcgtctttctacttctaaagcattattagacatttacaataataagtcagtagataatgctattgttaaagtctatggtaaaggtaagaaacttattataacaggattttatctcaaacaaaatatgatacgttatgttattgagtggataggggatgattttacaaacgatatatacaaaatgattaatttctataatgcgttattcggtaacgatgaattaaaaatagtatcctgtgaaaacactctatgcccgtttatagaacttggtagatgctattatggtaaaaaatgtaagtatatacacggagatcaatgtgatatctgtggtctatatatactacaccctaccgatattaaccaacgagtttctcacaagaaaacttgtttagtagatagagattctttgattgtgtttaaaagaagtaccagtaaaaagtgtggcatatgcatagaagaaataaacaaaaaacatatttccgaacagtattttggaattctcccaagttgtaaacatattttttgcctatcatgtataagacgttgggcagatactaccagaaatacagatactgaaaatacgtgtcctgaatgtagaatagtttttcctttcataatacccagtaggtattggatagataataaatatgataaaaaaatattatataatagatataagaaaatgatttttacaaaaatacctataagaacaataaaaatataattacatttacggaaaatagctggttttagtttaccaacttagagtaattatcatattgaatctatattgctaattagctaataaaaacccgggttaattaattagtcatcaggcagggcgagaacgagactatctgctcgttaattaattagagcttctttattctatacttaaaaagtgaaaataaatacaaaggttcttgagggttgtgttaaattgaaagcgagaaataatcataaattatttcattatcgcgatatccgttaagtttgtatcgtagcggccgccatggaaaagattgtgctgctgtttgctgtgattagcctggtgaagtcagatcagatttgtatcggttaccatgccaataattctactaaacaggtggatacaattatggaaaagaacgtgaccgtgacacacgctcaggacatcctggagagaactcataacgggaagctgtgcgatctgaatggtgtgaaacccctgatcctgaaggactgctctgtggcaggctggctgctgggaaaccccatgtgtgatgagttcatcagagtgcctgaatggtcctacattgtggagagggctaaccctgcaaatgatctgtgctacccaggaaccctgaacgactatgaggaactgaagcacctgctgagccgcatcaaccatttcgaaaagacactgatcatcccccggagctcctggcctaatcacgagactagcctgggagtgtccgcagcttgtccataccagggagcatcttcattctttcgcaacgtggtgtggctgatcaagaaaaatgatgcctaccccaccatcaaaatctcatacaacaacacaaaccgggaagatcttctgatcctgtggggcatccaccattccaacaatgcagccgagcagactaacctgtacaaaaatcctgatacctatgtgtctgtggggacttcaaccctgaaccagcgcctggtgccaaagatcgccactcggtcacaagtgaatgggcagagtggtcgcatggatttcttttggaccatcctgaagccaaacgacgctattcacttcgaaagcaacggcaattttatcgcccccgagtacgcttataagattgtgaagaaaggagacagtaccatcatgaaaagcgagatggaatacgggcactgcaacacaaagtgtcagactcctatcggtgccattaacagtagcatgccattccacaatatccatcccctgacaattggggagtgccccaagtatgtgaaatctaacaagctggtgctggctactggtctgagaaacagccccctgagagagacccggggcctgtttggagcaattgctgggtttattgagggcggatggcagggtatggtggatgggtggtacggttatcaccattccaacgaacaggggtctggttacgctgcagataaagagtccacacagaaggctattgacggagtgactaacaaagtgaacagcatcattgacaagatgaatactcagttcgaggcagtggggagagaatttaacaatctggagagaaggatcgaaaacctgaataagaaaatggaagatggcttcctggacgtgtggacctacaacgcagagctgctggtgctgatggagaatgaaaggacactggattttcacgacagcaacgtgaaaaatctgtatgataaagtgagactgcagctgagggacaacgctaaagaactgggcaatggatgtttcgagttttaccataagtgcgataacgagtgtatggaaagtgtgagaaatggcacatacgactatccaaaatatagcgaggaagcaatcctgaagagggaggaaattagcggcgtgaaactggagtccatcggaacctaccagatcctgtcaatttatagtacagtggcctcctctctggcactggccatcattgtggctgggctgtctctgtggatgtgtagtaacgggagtctgcagtgtaggatttgtatctgagcggccgcctcgagtttttattgactagttaatcataagataaataatatacagcattgtaaccatcgtcatccgttatacggggaataatattaccatacagtattattaaattttcttacgaagaatatagatcggtatttatcgttagtttattttacatttattaattaaacatgtctactattacctgttatggaaatgacaaatttagttatataatttatgataaaattaagataataataatgaaatcaaataattatgtaaatgctactagattatgtgaattacgaggaagaaagtttacgaactggaaaaaattaagtgaatctaaaatattagtcgataatgtaaaaaaaataaatgataaaactaaccagttaaaaacggatatgattatatacgttaaggatattgatcataaaggaagagatacttgcggttactatgtacaccaagatctggtatcttctatatcaaattggatatctccgttattcgccgttaaggtaaataaaattattaactattatatatgtaatgaatatgatatacgacttagcgaaatggaatctgatatgacagaagtaatagatgtagttgataaattagtaggaggatacaatgatgaaatagcagaaataatatatttgtttaataaatttatagaaaaatatattgctaacatatcgttatcaactgaattatctagtatattaaataattttataaattttaataaaaaatacaataacgacataaaagatattaaatctttaattcttgatctgaaaaacacatctataaaactagataaaaagttattcgataaagataataatgaatcgaacgatgaaaaattggaaacagaagttgataagctaatttttttcatctaaatagtattattttattgaagtacgaagttttacgttagataaataataaaggtcgatttttattttgttaaatatcaaatatgtcattatctgataaagatacaaaaacacacggtgattatcaaccatctaacgaacagatattacaaaaaatacgtcggactatggaaaacgaagctgatagcctcaatagaagaagcattaaagaaattgttgtagatgttatgaagaattgggatcatcctctcaacgaagaaatagataaagttctaaactggaaaaatgatacattaaacgatttagatcatctaaatacagatgataatattaaggaaatcatacaatgtctgattagagaatttgcgtttaaaaagatcaattctattatgtatagttatgctatggtaaaactcaattcagataacgaaacattgaaagataaaattaaggattattttatagaaactattcttaaagacaaacgtggttataaacaaaagccattaccc

SEQ ID NO: 13 - DNA, 4754 bp, artificial
  Nucleotide sequence of donor plasmid  pF8 H6p3Mut-HA H5N2
  Flanking Arms (1)..(1429)
  H6 Promoter (1516)..(1639)
  Mut-HA H5N2 (1649)..(3343)
  Flanking Arms (3379)..(4754)
gaccctttacaagaataaaagaagaaacaactgtgaaatagtttataaatgtaattcgtatgcagaaaacgataatatattttggtatgagaaatctaaaggagacatagtttgtatagacatgcgctcttccgatgagatattcgatgcttttctaatgtatcatatagctacaagatatgcctatcatgatgatgatatatatctacaaatagtgttatattattctaataatcaaaatgttatatcttatattacgaaaaataaatacgttaagtatataagaaataaaactagagacgatattcataaagtaaaaatattagctctagaagactttacaacggaagaaatatattgttggattagtaatatataacagcgtagctgcacggttttgatcattttccaacaatataaaccaatgaaggaggacgactcatcaaacataaataacattcacggaaaatattcagtatcagatttatcacaagatgattatgttattgaatgtatagacggatcttttgattcgatcaagtatagagatataaaggttataataatgaagaataacggttacgttaattgtagtaaattatgtaaaatgcggaataaatacttttctagatggttgcgtctttctacttctaaagcattattagacatttacaataataagtcagtagataatgctattgttaaagtctatggtaaaggtaagaaacttattataacaggattttatctcaaacaaaatatgatacgttatgttattgagtggataggggatgattttacaaacgatatatacaaaatgattaatttctataatgcgttattcggtaacgatgaattaaaaatagtatcctgtgaaaacactctatgcccgtttatagaacttggtagatgctattatggtaaaaaatgtaagtatatacacggagatcaatgtgatatctgtggtctatatatactacaccctaccgatattaaccaacgagtttctcacaagaaaacttgtttagtagatagagattctttgattgtgtttaaaagaagtaccagtaaaaagtgtggcatatgcatagaagaaataaacaaaaaacatatttccgaacagtattttggaattctcccaagttgtaaacatattttttgcctatcatgtataagacgttgggcagatactaccagaaatacagatactgaaaatacgtgtcctgaatgtagaatagtttttcctttcataatacccagtaggtattggatagataataaatatgataaaaaaatattatataatagatataagaaaatgatttttacaaaaatacctataagaacaataaaaatataattacatttacggaaaatagctggttttagtttaccaacttagagtaattatcatattgaatctatattgctaattagctaataaaaacccgggttaattaattagtcatcaggcagggcgagaacgagactatctgctcgttaattaattagagcttctttattctatacttaaaaagtgaaaataaatacaaaggttcttgagggttgtgttaaattgaaagcgagaaataatcataaattatttcattatcgcgatatccgttaagtttgtatcgtagcggccgccatggaaaagattgtgctgctgtttgctgtgatttccctggtgaagtccgaccagatttgtattggctaccacgctaataactcaaccaaacaggtggatacaattatggaaaagaacgtgaccgtgacacacgctcaggacatcctggagagaactcataacgggaagctgtgcgatctgaatggtgtgaaacccctgatcctgaaggactgctcagtggcaggctggctgctgggaaaccccatgtgtgatgagttcatcagagtgcctgaatggtcctacattgtggagagggctaaccctgcaaatgatctgtgctacccaggaaccctgaacgactatgaggaactgaagcacctgctgagtcgcatcaaccatttcgaaaagacactgatcatcccccggaacagctggcctaatcacgagacttcactgggcgtgagtgccgcttgtccataccagggagcaagctccttctttcgcaacgtggtgtggctgatcaagaaaaacaatgcctaccccaccatcaaaatctcctacaacaacacaaatcgggaagatcttctgatcctgtggggcatccaccattctaacaatgcagccgagcagactaacctgtacaaaaatcctgacacctatgtgagcgtggggacttccaccctgaaccagcgcctggtgccaaagatcgccactcggtctcaggtgaacgggcagaatggtcgcatggatttcttttggaccatcctgaagccaaatgacgctattcacttcgaatccaacggcaattttatcgcccccgagtacgcttataagattgtgaagaaaggagactctaccatcatgaaatcagagatggaatacgggcactgcaacacaaagtgtcagactcctatcggtgccattaactcttcaatgccattccacaatatccatcccctgacaattggggagtgccccaagtatgtgaaatcaaacaagctggtgctggctactggtctgaggaatagtcctctgcgcgaaacccggggcctgtttggagcaattgctggttttattgagggcggatggcagggtatggtggatgggtggtacggttatcaccatagtaacgaacaggggagcggttacgctgcagataaagagtctacacagaaggctattgacggagtgactaacaaagtgaacagcatcattgacaagatgaacactcagttcgaggcagtggggagagaatttaacaatctggagagaaggatcgaaaacctgaataagaaaatggaagatggcttcctggacgtgtggacctacaacgcagagctgctggtgctgatggagaatgaaaggacactggattttcacgacagcaacgtgaaaaatctgtatgataaagtgagactgcagctgagggacaacgctaaagaactgggcaatggatgtttcgagttttaccataagtgcgataacgagtgtatggaaagcgtgagaaatggcacatacgactatccaaaatattccgaggaagcaatcctgaagagggaggaaatttccggcgtgaaactggagtctatcggaacctaccagatcctgtccatttattctacagtggccagtagcctggcactggccatcattgtggctggtctgtctctgtggatgtgttcaaacggtagtctgcagtgtagaatctgtatctgagcggccgcctcgagtttttattgactagttaatcataagataaataatatacagcattgtaaccatcgtcatccgttatacggggaataatattaccatacagtattattaaattttcttacgaagaatatagatcggtatttatcgttagtttattttacatttattaattaaacatgtctactattacctgttatggaaatgacaaatttagttatataatttatgataaaattaagataataataatgaaatcaaataattatgtaaatgctactagattatgtgaattacgaggaagaaagtttacgaactggaaaaaattaagtgaatctaaaatattagtcgataatgtaaaaaaaataaatgataaaactaaccagttaaaaacggatatgattatatacgttaaggatattgatcataaaggaagagatacttgcggttactatgtacaccaagatctggtatcttctatatcaaattggatatctccgttattcgccgttaaggtaaataaaattattaactattatatatgtaatgaatatgatatacgacttagcgaaatggaatctgatatgacagaagtaatagatgtagttgataaattagtaggaggatacaatgatgaaatagcagaaataatatatttgtttaataaatttatagaaaaatatattgctaacatatcgttatcaactgaattatctagtatattaaataattttataaattttaataaaaaatacaataacgacataaaagatattaaatctttaattcttgatctgaaaaacacatctataaaactagataaaaagttattcgataaagataataatgaatcgaacgatgaaaaattggaaacagaagttgataagctaatttttttcatctaaatagtattattttattgaagtacgaagttttacgttagataaataataaaggtcgatttttattttgttaaatatcaaatatgtcattatctgataaagatacaaaaacacacggtgattatcaaccatctaacgaacagatattacaaaaaatacgtcggactatggaaaacgaagctgatagcctcaatagaagaagcattaaagaaattgttgtagatgttatgaagaattgggatcatcctctcaacgaagaaatagataaagttctaaactggaaaaatgatacattaaacgatttagatcatctaaatacagatgataatattaaggaaatcatacaatgtctgattagagaatttgcgtttaaaaagatcaattctattatgtatagttatgctatggtaaaactcaattcagataacgaaacattgaaagataaaattaaggattattttatagaaactattcttaaagacaaacgtggttataaacaaaagccattaccc

SEQ ID NO: 14 - protein, 7 aa, artificial
  highly pathogenic HA cleavage site
RERRRKR

SEQ ID NO: 15 - protein, 4 aa, artificial
  low pathogenic HA cleavage site
RETR

SEQ ID NO: 16 - DNA, 1412 bp, artificial
  mCMV promoter
gaattcactagtggatcccccaactccgcccgttttatgactagaaccaatagtttttaatgccaaatgcactgaaatcccctaatttgcaaagccaaacgccccctatgtgagtaatacggggactttttacccaatttcccaagcggaaagccccctaatacactcatatggcatatgaatcagcacggtcatgcactctaatggcggcccatagggactttccacatagggggcgttcaccatttcccagcataggggtggtgactcaatggcctttacccaagtacattgggtcaatgggaggtaagccaatgggtttttcccattactggcaagcacactgagtcaaatgggactttccactgggttttgcccaagtacattgggtcaatgggaggtgagccaatgggaaaaacccattgctgccaagtacactgactcaatagggactttccaatgggtttttccattgttggcaagcatataaggtcaatgtgggtgagtcaatagggactttccattgtattctgcccagtacataaggtcaatagggggtgaatcaacaggaaagtcccattggagccaagtacactgcgtcaatagggactttccattgggttttgcccagtacataaggtcaataggggatgagtcaatgggaaaaacccattggagccaagtacactgactcaatagggactttccattgggttttgcccagtacataaggtcaatagggggtgagtcaacaggaaagtcccattggagccaagtacattgagtcaatagggactttccaatgggttttgcccagtacataaggtcaatgggaggtaagccaatgggtttttcccattactggcacgtatactgagtcattagggactttccaatgggttttgcccagtacataaggtcaataggggtgaatcaacaggaaagtcccattggagccaagtacactgagtcaatagggactttccattgggttttgcccagtacaaaaggtcaatagggggtgagtcaatgggtttttcccattattggcacgtacataaggtcaataggggtgagtcattgggtttttccagccaatttaattaaaacgccatgtactttcccaccattgacgtcaatgggctattgaaactaatgcaacgtgacctttaaacggtactttcccatagctgattaatgggaaagtaccgttctcgagccaatacacgtcaatgggaagtgaaagggcagccaaaacgtaacaccgccccggttttcccctggaaattccatattggcacgcattctattggctgagctgcgttctacgtgggtataagaggcgcgaccagcgtcggtaccgtcgcagtcttcggtctgaccaccgtagaacgcagagctcctcgctgcag

SEQ ID NO: 17 - DNA, 1692 bp, artificial
  17   DNA encoding mutant H5N2 HA in plasmid pCD046-H5N2 HA (rHVT510), wild-type
atggagaaaatagtgcttctttttgcagtgattagccttgttaaaagtgatcagatttgcattggttaccatgcaaacaactcaacaaagcaggttgacacgataatggagaaaaacgtcactgttacacatgcccaagacatactggaaaggacacacaacgggaagctctgcgatcttaatggagtgaaacccctgattctaaaggattgtagcgtagctgggtggctccttggaaatccaatgtgcgacgagttcatcagggtaccggaatggtcttacatcgtggagagggctaacccagccaacgacctctgttacccagggaccctcaatgactatgaggaactgaaacacctattgagcagaataaatcattttgagaaaactctgatcatccccaggagttcttggcccaatcatgaaacatcattaggggtgagcgcagcatgtccataccagggagcatcctcatttttcagaaatgtggtatggctcatcaaaaagaacgatgcatacccgacaataaagataagctacaataataccaatcgggaagatcttttgatactgtgggggattcatcattccaacaatgcagcagagcagacaaatctctataaaaacccagacacttatgtttccgttgggacatcaacattaaaccagagattggtgccaaaaatagctactagatcccaagtaaacgggcagagtggaagaatggatttcttctggacaattttaaaaccgaatgatgcaatccactttgagagtaatggaaatttcattgctccagaatatgcatacaaaattgtcaagaaaggggactcaacaattatgaaaagtgaaatggagtatggccactgcaacaccaaatgtcaaactccaataggggcgataaactctagcatgccattccacaatatacaccctctcaccatcggggaatgccccaaatacgtgaagtcaaacaaattagtccttgcgactgggctcagaaatagtcctctaagagaaacgagaggactatttggagctatagcagggtttatagagggaggatggcagggaatggtagacggttggtatgggtatcatcatagcaatgagcaggggagtgggtacgctgcagacaaagaatcaacccaaaaggcaatagatggagttaccaataaggtcaactcaatcattgacaaaatgaacactcaatttgaggccgttggaagggaatttaataacttagaaaggagaatagagaatttaaacaagaaaatggaagacggattcctagatgtctggacttataatgctgaacttttagttctcatggaaaatgagagaactctagatttccatgactcaaatgtcaagaacctttacgacaaagtccgactacagcttagggataatgcaaaggagctgggtaatggttgtttcgagttctatcataaatgtgataacgaatgtatggagagcgtaagaaatgggacgtatgactaccctaagtattcagaagaagcaatattaaaaagagaagaaataagcggagtgaaattagaatcaataggaacttaccagatactgtcaatttattcaacagtggcgagttccctagcactggcaatcatagtggctggtctatctttatggatgtgctctaatgggtcgttacaatgcagaatttgcatc

SEQ ID NO: 18 - DNA, 218 bp, artificial
  SV40 PolyA tail
ggggatccagacatgataagatacattgatgagtttggacaaaccacaactagaatgcagtgaaaaaaatgctttatttgtgaaatttgtgatgctattgctttatttgtaaccattataagctgcaataaacaagttaacaacaacaattgcattcattttatgtttcaggttcagggggaggtgtgggaggttttttcggatcctctagagtcgac

SEQ ID NO: 19 - DNA, 5415 bp, artificial
  Nucleotide sequence of donor plasmid pCD046-H5N2 HA
  Recombination flanking arm (1)..(1241)
  mCMV promoter (1242)..(2653)
  H5N2 HA (2663)..(4357)
  SV40 polyA (4366)..(4583)
  Recombination flanking arm (4584)..(5415)
gagctcagggtatgatactcagctgttattgtggccgaccaggaggactccaatgcttagcattcataagaacgctagagatgctatttaacgatgtgctgtcgtctaaagaatttgtgcatttagcctttaaatgtaaaaccaatgacgcattcactacgctcgtgcgtgcaatttctgggccagggtatgcatattccataacagaaatcgacacttgagaagaggatctgactgtttgggataaaggtcgtttgggtctgtcctagcgatataatttatatgacgatatacattaaacatctgtgtgcagtacttaggtatttaatcatgtcgatgaaatgttatgtgtaaatatcggacaatatagataacgggcacgctgctattgtaacgtgcgcccgcgcgctagtgctgactaatagtgtggatgatgtatacagtatattacaaacggaaatgatacgtaataaattatgtactcttattgatttataaaaacatacatgcagtgttgctatgtcacataattagcctcgcccgtctacgctccactgaagataatgggctcccgctgttcaaaaaaatcagcgtgcgtcgataagactttggtgcagtctcttcggggtcgcaatttagatttgccgcatggagggtatctggggatttttgccaatgctggagcgacgactgtacgattcgtcccatcgggatctagcagaccaatgatgttgacacacatcggccatgcatgtacggacggtctattgcgcgagtttgttattttcgaaggacaagatggaagtgtatatggaaccgacaataatgttagtttgcatttcttagggcggaatctacatgatatcttatccaagcggggtatgagccagagagatgtgatggtcataaagggtaaattttttagatctgaaataacgcagttgcccaaacaacgatcgcgattaaaagaaaaatcggatggttcaattaggacatgcatggattctgtgcgcataaaccataaccgcagcactgttgggcacttcggtaactcaaatgcgaagcgttgcacgtctgcgataactacgcctactatgcacattgttactcctgcatcttaaaaatatatcctgtagtaattttcacagcaatgtcataacatcatctcgctaaagaatgacctgggattggagaagtaatgaatatttgcaaccaatgcattgaataaactaacattaaacgaattcactagtggatcccccaactccgcccgttttatgactagaaccaatagtttttaatgccaaatgcactgaaatcccctaatttgcaaagccaaacgccccctatgtgagtaatacggggactttttacccaatttcccaagcggaaagccccctaatacactcatatggcatatgaatcagcacggtcatgcactctaatggcggcccatagggactttccacatagggggcgttcaccatttcccagcataggggtggtgactcaatggcctttacccaagtacattgggtcaatgggaggtaagccaatgggtttttcccattactggcaagcacactgagtcaaatgggactttccactgggttttgcccaagtacattgggtcaatgggaggtgagccaatgggaaaaacccattgctgccaagtacactgactcaatagggactttccaatgggtttttccattgttggcaagcatataaggtcaatgtgggtgagtcaatagggactttccattgtattctgcccagtacataaggtcaatagggggtgaatcaacaggaaagtcccattggagccaagtacactgcgtcaatagggactttccattgggttttgcccagtacataaggtcaataggggatgagtcaatgggaaaaacccattggagccaagtacactgactcaatagggactttccattgggttttgcccagtacataaggtcaatagggggtgagtcaacaggaaagtcccattggagccaagtacattgagtcaatagggactttccaatgggttttgcccagtacataaggtcaatgggaggtaagccaatgggtttttcccattactggcacgtatactgagtcattagggactttccaatgggttttgcccagtacataaggtcaataggggtgaatcaacaggaaagtcccattggagccaagtacactgagtcaatagggactttccattgggttttgcccagtacaaaaggtcaatagggggtgagtcaatgggtttttcccattattggcacgtacataaggtcaataggggtgagtcattgggtttttccagccaatttaattaaaacgccatgtactttcccaccattgacgtcaatgggctattgaaactaatgcaacgtgacctttaaacggtactttcccatagctgattaatgggaaagtaccgttctcgagccaatacacgtcaatgggaagtgaaagggcagccaaaacgtaacaccgccccggttttcccctggaaattccatattggcacgcattctattggctgagctgcgttctacgtgggtataagaggcgcgaccagcgtcggtaccgtcgcagtcttcggtctgaccaccgtagaacgcagagctcctcgctgcaggcggccgccatggagaaaatagtgcttctttttgcagtgattagccttgttaaaagtgatcagatttgcattggttaccatgcaaacaactcaacaaagcaggttgacacgataatggagaaaaacgtcactgttacacatgcccaagacatactggaaaggacacacaacgggaagctctgcgatcttaatggagtgaaacccctgattctaaaggattgtagcgtagctgggtggctccttggaaatccaatgtgcgacgagttcatcagggtaccggaatggtcttacatcgtggagagggctaacccagccaacgacctctgttacccagggaccctcaatgactatgaggaactgaaacacctattgagcagaataaatcattttgagaaaactctgatcatccccaggagttcttggcccaatcatgaaacatcattaggggtgagcgcagcatgtccataccagggagcatcctcatttttcagaaatgtggtatggctcatcaaaaagaacgatgcatacccgacaataaagataagctacaataataccaatcgggaagatcttttgatactgtgggggattcatcattccaacaatgcagcagagcagacaaatctctataaaaacccagacacttatgtttccgttgggacatcaacattaaaccagagattggtgccaaaaatagctactagatcccaagtaaacgggcagagtggaagaatggatttcttctggacaattttaaaaccgaatgatgcaatccactttgagagtaatggaaatttcattgctccagaatatgcatacaaaattgtcaagaaaggggactcaacaattatgaaaagtgaaatggagtatggccactgcaacaccaaatgtcaaactccaataggggcgataaactctagcatgccattccacaatatacaccctctcaccatcggggaatgccccaaatacgtgaagtcaaacaaattagtccttgcgactgggctcagaaatagtcctctaagagaaacgagaggactatttggagctatagcagggtttatagagggaggatggcagggaatggtagacggttggtatgggtatcatcatagcaatgagcaggggagtgggtacgctgcagacaaagaatcaacccaaaaggcaatagatggagttaccaataaggtcaactcaatcattgacaaaatgaacactcaatttgaggccgttggaagggaatttaataacttagaaaggagaatagagaatttaaacaagaaaatggaagacggattcctagatgtctggacttataatgctgaacttttagttctcatggaaaatgagagaactctagatttccatgactcaaatgtcaagaacctttacgacaaagtccgactacagcttagggataatgcaaaggagctgggtaatggttgtttcgagttctatcataaatgtgataacgaatgtatggagagcgtaagaaatgggacgtatgactaccctaagtattcagaagaagcaatattaaaaagagaagaaataagcggagtgaaattagaatcaataggaacttaccagatactgtcaatttattcaacagtggcgagttccctagcactggcaatcatagtggctggtctatctttatggatgtgctctaatgggtcgttacaatgcagaatttgcatctaagcggccgcggggatccagacatgataagatacattgatgagtttggacaaaccacaactagaatgcagtgaaaaaaatgctttatttgtgaaatttgtgatgctattgctttatttgtaaccattataagctgcaataaacaagttaacaacaacaattgcattcattttatgtttcaggttcagggggaggtgtgggaggttttttcggatcctctagagtcgacaattattttatttaataacatatagcccaaagacctctatgaacatttagtttcccgtatactcaacggcgcgtgtacacacgcatctctttgcatagcgatgaagtttgttcggcagcagaaaatgcagatatccaacaatctggagaaaacttatcatcacagtggcagtggaaacataccccctctatattcatggtataattatcgtctacagcgtccaggatagtggcgtgagaaaatggagatctgcagccctcctttccatggcatgccgctttattgttcattaaacgcacaatggtctcaacgccagatatgggcatagattctgaagaacccgttgacaatccgaagaagaaggcgtgcaggtctttggaagactcgcacgttggtcttataatgtatgatcgagatgtcaccctaatgccacatggtacaggcttatcgcggtcatggcgatcggacttgtaatttgcaacgatgggcaaaggatcgacgacatgccaaacattctgaacccgtagagatgttaacgatgacgaggatgaatatcccatgctcgctgccatagtatcaagtacaccgcgaataaggacgcgtccaacatcgttatatgcacacaatgggctacacgtgactaacacccccgaatattagtcatatgtgagtttcagtctggctcccatatagcctgtagactatttgtggtttaagtgtgaacgaggcgctgtgaacgagactcgggccgattgtaagaacaagcaaatgcactttccatttaacaagaagtgtagagagaatactcaacctctttggatgtatcctcgag

SEQ ID NO: 20 - protein, 564 aa, artificial
  ALT19477  with modified low pathogenic cleave site hemagglutinin [Influenza A virus (A/wood /Oregon/AH0007263/2015(H5N2))]
MEKIVLLFAVISLVKSDQICIGYHANNSTKQVDTIMEKNVTVTHAQDILEKTHNGKLCDLNGVKPLILKDCSVAGWLLGNPMCDEFIRIPEWSYIVERANPANDLCYPGTLNDYEELKHLLSRINHFEKTLIIPRSSWPNHETSLGVSAACPYQGASSFFRNVVWLIKKNDAYPTIKISYNNTNREDLLILWGIHHSNNAAEQTNLYKNPDTYVSVGTSTLNQRLVPKIATRSQVNGQSGRMDFFWTILKPNDAIHFESNGNFIAPEYAYKIVKKGDSTIMKSEMEYGHCNTKCQTPIGAINSSMPFHNIHPLTIGECPKYVKSNKLVLATGLRNSPLRETRGLFGAIAGFIEGGWQGMVDGWYGYHHSNEQGSGYAADKESTQKAIDGVTNKVNSIIDKMNTQFEAVGREFNNLERRIENLNKKMEDGFLDVWTYNAELLVLMENERTLDFHDSNVKNLYDKVRLQLRDNAKELGNGCFEFYHKCDNECMESVRNGTYDYPKYSEEAILKREEISGVKLESIGTYQILSIYSTVASSLALAIIVAGLSLWMCSNGSLQCRICI

SEQ ID NO: 21 - protein, 564 aa, artificial
  ALT19381 with modified low pathogenic  cleave site hemagglutinin [Influenza A virus A/mallard/Idaho/AH0007413/2015(H5N2))]
MEKIVLLFAVISLVKSDQICIGYHANNSTKQVDTIMEKNVTVTHAQDILEKTHNGKLCDLNGVKPLILKDCSVAGWLLGNPMCDEFIRVPEWSYIVERANPANDLCYPGTLNDYEELKHLLSRINHFEKTLIIPRSSWPNHETSLGVSAACPYQGASSFFRNVVWLIKKNDAYPTIKISYNNTNREDLLILWGIHHSNNAAEQTNLYKNPDTYVSVGTSTLNQRLVPKIATRSQVNGQSGRMDFFWTILKPNDAIHFESNGNFIAPEYAYKIVKKGDSTIMKSEMEYGHCNTKCQTPIGAINSSMPFHNIHPLTIGECPKYVKSNKLVLATGLRNSPLRETRGLFGAIAGFIEGGWQGMVDGWYGYHHSNEQGSGYAADKESTQKAIDGVTNKVNSIIDKMNTQFEAVGREFNNLERRIENLNKKMEDGFLDVWTYNAELLVLMENERTLDFHDSNVKNLYDKVRLQLKDNAKELGNGCFEFYHKCDNECMESVRNGTYDYPKYSEEAILKREEISGVKLESIGTYQILSIYSTVASSLALAIIVAGLSLWMCSNGSLQCRICI

SEQ ID NO: 22 - protein, 564 aa, artificial
  AKH14518 with modified low pathogenic  cleave site   564 aa hemagglutinin [Influenza A virusA/turkey/Minnesota/7172-1/2015(H5N2))]
MEEIVLLFAVISLVKSDQICIGYHANNSTKQVDTIMEKNVTVTHAQDILEKTHNGKLCDLNGVKPLILKDCSVAGWLLGNPMCDEFIRVPEWSYIVERANPANDLCYPGTLNDYEELKHLLSRINHFEKTLIIPRSSWPNHETSLGVSAACPYQGASSFFRNVVWLIKKNDAYPTIKISYNNTNREDLLILWGIHHSNNAAEQTNLYKNPDTYVSVGTSTLNQRLVPKIATRSQVNGQSGRMDFFWTILKPNDAIHFESNGNFIAPEYAYKIVKKGDSTIMKSEMEYGHCNTKCQTPIGAINSSMPFHNIHPLTIGECPKYVKSNKLVLATGLRNSPLRETRGLFGAIAGFIEGGWQGMVDGWYGYHHSNEQGSGYAADKESTQKAIDGVTNKVNSIIDKMNTQFEAVGREFNNLERRIENLNKKMEDGFLDVWTYNAELLVLMENERTLDFHDSNVKNLYDKVRLQLRDNAKELGNGCFEFYHKCDNECMESVRNGTYDYPKYSEEAILKREEISGVKLESIGTYQILSIYSTVASSLALAIIVAGLSLWMCSNGSLQCRICI

SEQ ID NO: 23 - protein, 564 aa, artificial
  ALH21333 with modified low pathogenic  cleave site 564 aa hemagglutinin [Influenza A virus (A/chicken/Montana/15-010559-1/2015(H5N2))]
MEKIVLLFAVVNLVKSDQICIGYHANNSTKQVDTIMEKNVTVTHAQDILEKTHNGKLCDLNGVKPLILKDCSVAGWLLGNPMCDEFIRVPEWSYIVERANPANDLCYPGTLNDYEELKHLLSRINHFEKTLIIPRSSWPNHETSLGVSAACPYQGASSFFRNVVWLIKKNDAYPTIKISYNNTNREDLLILWGIHHSNNAAEQTNLYKNPDTYVSVGTSTLNQRLVPKIATRSQVNGQSGRMDFFWTILKPNDAIHFESNGNFIAPEYAYKIVKKGDSTIMKSEMEYGHCNTKCQTPIGAINSSMPFHNIHPLTIGECPKYVKSNKLVLATGLRNSPLRETRGLFGAIAGFIEGGWQGMVDGWYGYHHSNEQGSGYAADKESTQKAIDGVTNKVNSIIDKMNTQFEAVGREFNNLERRIENLNKKMEDGFLDVWTYNAELLVLMENERTLDFHDSNVKNLYDKVRLQLRDNAKELGNGCFEFYHKCDNECMESVRNGTYDYPKYSEEAILKREEISGVKLESIGTYQILSIYSTVASSLALAIIVAGLSLWMCSNGSLQCRICI

SEQ ID NO: 24 - protein, 564 aa, artificial
  ALT19525 with modified low pathogenic  cleave site hemagglutinin [Influenza virus(A/mallard/Oregon/AH0003952/2015(H5N2))]
MEKIVLLFAVVSLVKSDQICIGYHANNSTKQVDTIMEKNVTVTHAQDILEKTHNGKLCDLNGVKPLILKDCSVAGWLLGNPMCDEFIRVPEWSYIVERANPANDLCYPGTLNDYEELKHLLSRINHFEKTLIIPRSSWPNHETSLGVSAACPYQGASSFFRNVVWLIKKNDAYPTIKISYNNTNREDLLILWGIHHSNNAAEQTNLYKNPDTYVSVGTSTLNQRLVPKIATRSQVNGQSGRMDFFWTILKPNDAIHFESNGNFIAPEYAYKIVKKGDSTIMKSEMEYGHCNTKCQTPIGAINSSMPFHNIHPLTIGECPKYVKSNKLVLATGLRNSPLRETRGLFGAIAGFIEGGWQGMVDGWYGYHHSNEQGSGYAADKESTQKAIDGVTNKVNSIIDKMNTQFEAVGREFNNLERRIENLNKKMEDGFLDVWTYNAELLVLMENERTLDFHDSNVKNLYDKVRLQLRDNAKELGNGCFEFYHKCDNECMESVRNGTYDYPKYSEEAILKREEISGVKLESIGTYQILSIYSTVASSLALAIIVAGLFLWMCSNGSLQCRICI

SEQ ID NO: 25 - protein, 564 aa, artificial
  AKN08877 with modified low pathogenic  cleave site hemagglutinin [Influenza A virus (A/chicken/Iowa/14589-1/2015(H5N2))]
MEKIVLPFAVISLVKSDQICIGYHANNSTKQVDTIMEKNVTVTHAQDILEKTHNGKLCDLNGVKPLILKDCSVAGWLLGNPICDEFIRVPEWSYIVERANPANDLCYPGTLNDYEELKHLLSRINHFEKTLIIPRSSWPNHETSLGVSAACPYQGAPSFFRNVVWLIKKNDAYPTIKISYNNTNREDLLILWGIHHSNNAAEQTNLYKNPDTYVSVGTSTLNQRLVPKIATRSQVNGQSGRMDFFWTILKPNDAIHFESNGNFIAPEYAYKIVKKGDSTIMKSEMEYGHCNTKCQTPIGAINSSMPFHNIHPLTIGECPKYVKSNKLVLATGLRNSPQRETRGLFGAIAGFIEGGWQGMVDGWYGYHHSNEQGSGYAADKESTQKAIDGVTNKVNSIIDKMNTQFEAVGREFNNLERRIENLNKKMEDGFLDVWTYNAELLVLMENERTLDFHDSNVKNLYDKVRLQLRDNAKELGNGCFEFYHKCDNECMESVRNGTYDYPKYSEEAILKREEISGVKLESIGTYQILSIYSTVASSLALAIIVAGLSLWMCSNGSLQCRICI

SEQ ID NO: 26 - protein, 564 aa, artificial
  AJS16153  with modified low pathogenic  cleave site hemagglutinin [Influenza A virus(A/duck/EasternChina/S0131/2014(H5N2))]
MEKIVLLLAIVSLVKSDQICIGYHANNSTKQVDTIMEKNVTVTHAQDILEKTHNGKLCDLNGVKPLILKDCSVAGWLLGNPMCDEFIRVPEWSYIVERANPANDLCYPGTLNDYEELKHLLSRINHFEKTLIIPKSSWPNHETSLGVSAACPYQGASSFFRNVVWLIKKNDAYPTIKISYNNTNREDLLILWGIHHSNNAAEQTNLYKNPDTYVSVGTSTLNQRLVPKIATRSQVNGQRGRMDFFWTILKPNDAIHFESNGNFIAPEYAYKIVKKGDSTIMKSEVEYGHCNTKCQTPIGAINSSMPFHNIHPLTIGECPKYVKSNKLVLATGLRNSPLRETRGLFGAIAGFIEGGWQGMVDGWYGYHHSNEQGSGYAADKESTQKAIDGVTNKVNSIIDKMNTQFEAVGREFNNLERRIENLNKKMEDGFLDVWTYNAELLVLMENERTLDFHDSNVKNLYDKVRLQLRDNAKELGNGCFEFYHKCDNECMESVRNGTYDYPQYSEEARLKREEISGVKLESIGTYQILSIYSTVASSLVLAIIVAGLSLWMCSNGSLQCRICI

SEQ ID NO: 27 - protein, 564 aa, artificial
  ALP30284 with modified low pathogenic  cleave site hemagglutinin [Influenza A virus (A/duck/Zhejiang/727041/2014(H5N2))]
MEKIVLLLAVVSLVKSDQICIGYHANNSTEQVDTIMEKNVTVTHAQDILEKTHNGKLCDLNGVKPLILKDCSVAGWLLGNPMCDEFIRVPEWSYIVERANPANDLCYPGNLNDYEELKHLLSRINHFEKTLIIPKSSWPNHETSLGVSAACPYQGMPSFFRNVVWLTKKNDAYPTIKMSYNNTNREDLLILWGIHHSNNAAEQTNLYKNPTTYVSVGTSTLNQRLVPKIATRSQVNGQRGRMDFFWTILKPKDAIHFESNGNFIAPEYAYKIVKKGDSTIMKSEIEYGHCNTKCQTPIGAINSSMPFHNIHPLTIGECPKYVKSNKLVLATGLRNSPLRETRGLFGAIAGFIEGGWQGMVDGWYGYHHSNEQGSGYAADRESTQKAIDGVTNKVNSIIDKMNTQFEAVGREFNNLERRIENLNKKMEDGFLDVWTYNAELLVLMENERTLDFHDSNVKNLYDKVRLQLRDNAKELGNGCFEFYHKCDNECMESVRNGTYDYPQYSEEARLKREEISGVKLESIGTYQILSIYSTVASSLALAIIVAGLSLWMCSNGSLQCRICI

SEQ ID NO: 28 - protein, 564 aa, artificial
  ALP30234 with modified low pathogenic  cleave site hemagglutinin [Influenza A virus(A/chicken/Zhejiang/727079/2014(H5N2))]
MEKIVLLLAVVSLVKSDQICIGYHANNSTEQVDTIMEKNVTVTHAQDILEKTHNGKLCDLNGVKPLILKDCSVAGWLLGNPMCDEFIRVPEWSYIVERANPANDLCYPGNLNDYEELKHLLSRINHFEKTLIIPKSSWPNHETSLGVSAACPYQGMPSFFRNVVWLTKKNDAYPTIKMSYNNTNREDLLILWGIHHSNNAAEQTNLYKNPTTYVSVGTSTLNQRLVPKIATRSQVNGQRGRMDFFWTILKPNDAIHFESNGNFIAPEYAYKIVKKGDSTIMKSEMEYGHCNTKCQTPIGAINSSMPFHNIHPLTIGECPKYVKSNKLVLATGLRNSPLRETRGLFGAIAGFIEGGWQGMVDGWYGYHHSNEQGSGYAADRESTQKAIDGVTNKVNSIIDKMNTQFEAVGREFNNLERRIENLNKKMEDGFLDVWTYNAELLVLMENERTLDFHDSNVKNLYDKVRLQLRDNAKELGNGCFEFYPKCDNECMESVRNGTYDYPQYSEEARLKREEISGVKLESIGTYQILSIYSTVASSLALAIIVAGLSLWMCSNGSLQCRICI